European Patent Application EP 4 582 450 A1, published July 9, 2025. Title: ANTI-PVRIG ANTIBODY AND APPLICATION THEREOF. Applicant: CSPC Megalith Biopharmaceutical Co., Ltd. Application WO. The sequence listing filed with the application follows.

SEQUENCE LISTING (55 sequences)

SEQ ID NO: 1 - protein, 5 aa, synthetic construct
SYWMH

SEQ ID NO: 2 - protein, 17 aa, synthetic construct
EINPSNGLTNYNEQFRN

SEQ ID NO: 3 - protein, 11 aa, synthetic construct
HHGSTYYALDS

SEQ ID NO: 4 - protein, 17 aa, synthetic construct
KSSQSLLNSINQKNFLA

SEQ ID NO: 5 - protein, 7 aa, synthetic construct
FASTRES

SEQ ID NO: 6 - protein, 9 aa, synthetic construct
QQHYSTPPT

SEQ ID NO: 7 - protein, 120 aa, synthetic construct
QVQLQQPGAELVKPGASVKLSCKASGYSFPSYWMHWVRQRPGQDLEWIGEINPSNGLTNYNEQFRNKATLTVDKSSSTAYMQLSSLTSEDSAVYYCARHHGSTYYALDSWGQGTSITVSS

SEQ ID NO: 8 - protein, 113 aa, synthetic construct
DIVMTQSPSSLAMSVGQKVTMSCKSSQSLLNSINQKNFLAWYQQRPGQSPKLLVYFASTRESGVPDRFIGSGSGTDFTLTISSVQAEDLADYFCQQHYSTPPTFGGGTKLEIK

SEQ ID NO: 9 - protein, 120 aa, synthetic construct
QVQLVQSGAEVKKPGASVKVSCKASGYSFPSYWMHWVRQAPGQGLEWMGEINPSNGLTNYNEQFRNRVTMTRDTSTSTVYMELSSLRSEDTAVYYCARHHGSTYYALDSWGQGTLVTVSS

SEQ ID NO: 10 - protein, 120 aa, synthetic construct
QVQLVQSGAEVKKPGASVKVSCKASGYSFPSYWMHWVRQAPGQGLEWIGEINPSNGLTNYNEQFRNRVTMTVDTSTSTVYMELSSLRSEDTAVYYCARHHGSTYYALDSWGQGTLVTVSS

SEQ ID NO: 11 - protein, 120 aa, synthetic construct
QVQLVQSGAEVKKPGASVKVSCKASGYSFPSYWMHWVRQAPGQGLEWIGEINPSNGLTNYNEQFRNRATMTVDTSTSTVYMELSSLRSEDTAVYYCARHHGSTYYALDSWGQGTLVTVSS

SEQ ID NO: 12 - protein, 120 aa, synthetic construct
QVQLVQSGAEVKKPGASVKVSCKASGYSFPSYWMHWVRQAPGQGLEWIGEINPSNGLTNYNEQFRNRATMTVDTSSSTVYMELSSLRSEDTAVYYCARHHGSTYYALDSWGQGTLVTVSS

SEQ ID NO: 13 - protein, 113 aa, synthetic construct
DIVMTQSPDSLAVSLGERATINCKSSQSLLNSINQKNFLAWYQQKPGQPPKLLIYFASTRESGVPDRFSGSGSGTDFTLTISSLQAEDVAVYYCQQHYSTPPTFGGGTKLEIK

SEQ ID NO: 14 - protein, 113 aa, synthetic construct
DIVMTQSPDSLAVSLGERATINCKSSQSLLNSINQKNFLAWYQQKPGQPPKLLVYFASTRESGVPDRFSGSGSGTDFTLTISSLQAEDVAVYFCQQHYSTPPTFGGGTKLEIK

SEQ ID NO: 15 - protein, 113 aa, synthetic construct
DIVMTQSPDSLAVSLGERATINCKSSQSLLNSINQKNFLAWYQQRPGQPPKLLVYFASTRESGVPDRFSGSGSGTDFTLTISSLQAEDVAVYFCQQHYSTPPTFGGGTKLEIK

SEQ ID NO: 16 - protein, 113 aa, synthetic construct
DIVMTQSPDSLAVSLGERATMSCKSSQSLLNSINQKNFLAWYQQRPGQPPKLLVYFASTRESGVPDRFSGSGSGTDFTLTISSLQAEDVAVYFCQQHYSTPPTFGGGTKLEIK

SEQ ID NO: 17 - protein, 5 aa, synthetic construct
NNFIE

SEQ ID NO: 18 - protein, 17 aa, synthetic construct
VINPGSGDANYNEKFKG

SEQ ID NO: 19 - protein, 17 aa, synthetic construct
VINPGSGDANYNEKFQG

SEQ ID NO: 20 - protein, 17 aa, synthetic construct
VINPGSGDANYAQKFQG

SEQ ID NO: 21 - protein, 5 aa, synthetic construct
HWLAY

SEQ ID NO: 22 - protein, 17 aa, synthetic construct
KSSQSLLSSGNQKNYLA

SEQ ID NO: 23 - protein, 17 aa, synthetic construct
RSSQSLLSSGNQKNYLS

SEQ ID NO: 24 - protein, 7 aa, synthetic construct
GASTRES

SEQ ID NO: 25 - protein, 7 aa, synthetic construct
GASTRET

SEQ ID NO: 26 - protein, 9 aa, synthetic construct
QNGHFYPYT

SEQ ID NO: 27 - protein, 114 aa, synthetic construct
QVQLQQSGAELVRPGTSVKVSCKASGYAFINNFIEWVKQRPGQGLEWIGVINPGSGDANYNEKFKGKATLTADKSSTTAYIQLSSLTSDDSAVYFCASHWLAYWGQGTLVTVSA

SEQ ID NO: 28 - protein, 113 aa, synthetic construct
DIVMTQSPSSLSVSAGEKVTMSCKSSQSLLSSGNQKNYLAWYQQKPGQPPKLLIYGASTRESGVPDRFTGSGSGTDFTLTISSVQAEDLAVYYCQNGHFYPYTFGGGTKLEIK

SEQ ID NO: 29 - protein, 114 aa, synthetic construct
QVQLVQSGAEVKKPGASVKVSCKASGYAFINNFIEWVRQAPGQGLEWIGVINPGSGDANYNEKFKGRATLTADKSITTAYIELSRLRSDDTAVYYCASHWLAYWGQGTTVTVSS

SEQ ID NO: 30 - protein, 114 aa, synthetic construct
QVQLVQSGAEVKKPGASVKVSCKASGYAFINNFIEWVRQAPGQGLEWIGVINPGSGDANYNEKFQGRVTLTADKSISTAYIELSRLRSDDTAVYYCASHWLAYWGQGTTVTVSS

SEQ ID NO: 31 - protein, 114 aa, synthetic construct
QVQLVQSGAEVKKPGASVKVSCKASGYAFINNFIEWVRQAPGQGLEWMGVINPGSGDANYNEKFQGRVTMTADTSISTAYMELSRLRSDDTAVYYCASHWLAYWGQGTTVTVSS

SEQ ID NO: 32 - protein, 114 aa, synthetic construct
QVQLVQSGAEVKKPGASVKVSCKASGYTFINNFIEWVRQAPGQGLEWMGVINPGSGDANYAQKFQGRVTMTRDTSISTAYMELSRLRSDDTAVYYCASHWLAYWGQGTTVTVSS

SEQ ID NO: 33 - protein, 113 aa, synthetic construct
EIVMTQSPPTLSVSPGERVTMSCKSSQSLLSSGNQKNYLAWYQQKPGQAPRLLIYGASTRESGVPDRFSGSGSGTDFTLTISSVQPEDFAVYYCQNGHFYPYTFGGGTKLEIK

SEQ ID NO: 34 - protein, 113 aa, synthetic construct
EIVMTQSPPTLSLSPGERVTLSCKSSQSLLSSGNQKNYLAWYQQKPGQAPRLLIYGASTRESGIPARFSGSGSGTDFTLTISSLQPEDFAVYYCQNGHFYPYTFGGGTKLEIK

SEQ ID NO: 35 - protein, 113 aa, synthetic construct
EIVMTQSPPTLSLSPGERVTLSCRSSQSLLSSGNQKNYLSWYQQKPGQAPRLLIYGASTRETGIPARFSGSGSGTDFTLTISSLQPEDFAVYYCQNGHFYPYTFGGGTKLEIK

SEQ ID NO: 36 - protein, 6 aa, synthetic construct
SDYAWN

SEQ ID NO: 37 - protein, 16 aa, synthetic construct
YIRYNGNTNYNPSLKS

SEQ ID NO: 38 - protein, 10 aa, synthetic construct
IYYDYDGFVY

SEQ ID NO: 39 - protein, 11 aa, synthetic construct
RASQNVYENLH

SEQ ID NO: 40 - protein, 7 aa, synthetic construct
FASDSIS

SEQ ID NO: 41 - protein, 9 aa, synthetic construct
LQLYSTPYT

SEQ ID NO: 42 - protein, 119 aa, synthetic construct
DVQLQESGPGLVKPSQSLSLTCTVTGYSITSDYAWNWIRQFPGNRLEWMGYIRYNGNTNYNPSLKSRISITRDTSKNQFFLQLNSVTTEDTATYYCAIIYYDYDGFVYWGQGTLVTVSA

SEQ ID NO: 43 - protein, 107 aa, synthetic construct
DILLTQSPATLSVTPGETVSLSCRASQNVYENLHWYQQKSHRSPRLLIKFASDSISGIPSRFTGSGSGTDYTLSINSVKPEDEGIYYCLQLYSTPYTFGGGTELEIK

SEQ ID NO: 44 - protein, 118 aa, synthetic construct
DVQLQESGPLVKPSETLSLTCTVTGYSITSDYAWNWIRQFPGKGLEWMGYIRYNGNTNYNPSLKSRITISRDTSKNQFSLKLSSVTAADTAVYYCAIIYYDYDGFVYWGQGTTVTVSS

SEQ ID NO: 45 - protein, 119 aa, synthetic construct
QVQLQESGPGLVKPSETLSLTCTVTGYSITSDYAWNWIRQPPGKGLEWMGYIRYNGNTNYNPSLKSRVTISVDTSKNQFSLKLSSVTAADTAVYYCAIIYYDYDGFVYWGQGTTVTVSS

SEQ ID NO: 46 - protein, 119 aa, synthetic construct
QVQLQESGPGLVKPSETLSLTCTVSGYSITSDYAWNWIRQPPGKGLEWIGYIRYNGNTNYNPSLKSRVTISVDTSKNQFSLKLSSVTAADTAVYYCAIIYYDYDGFVYWGQGTTVTVSS

SEQ ID NO: 47 - protein, 119 aa, synthetic construct
QVQLQESGPGLVKPSETLSLTCTVSGYSISSDYAWNWIRQPPGKGLEWIGYIRYNGNTNYNPSLKSRVTISVDTSKNQFSLKLSSVTAADTAVYYCAIIYYDYDGFVYWGQGTTVTVSS

SEQ ID NO: 48 - protein, 32 aa, synthetic construct
SSVQPEDFATYYCLQLYSTPYTFGGGTKLEIK

SEQ ID NO: 49 - protein, 107 aa, synthetic construct
DIQLTQSPSSLSASVGDRVTITCRASQNVYENLHWYQQKPGKAPKLLIKFASDSISGIPSRFSGSGSGTDYTLTISSLQPEDFATYYCLQLYSTPYTFGGGTKLEIK

SEQ ID NO: 50 - protein, 107 aa, synthetic construct
DIQMTQSPSSLSASVGDRVTITCRASQNVYENLHWYQQKPGKAPKLLIKFASDSISGVPSRFSGSGSGTDFTLTISSLQPEDFATYYCLQLYSTPYTFGGGTKLEIK

SEQ ID NO: 51 - protein, 330 aa, synthetic construct
ASTKGPSVFPLAPSSKSTSGGTAALGCLVKDYFPEPVTVSWNSGALTSGVHTFPAVLQSSGLYSLSSVVTVPSSSLGTQTYICNVNHKPSNTKVDKKVEPKSCDKTHTCPPCPAPELLGGPSVFLFPPKPKDTLMISRTPEVTCVVVDVSHEDPEVKFNWYVDGVEVHNAKTKPREEQYNSTYRVVSVLTVLHQDWLNGKEYKCKVSNKALPAPIEKTISKAKGQPREPQVYTLPPSREEMTKNQVSLTCLVKGFYPSDIAVEWESNGQPENNYKTTPPVLDSDGSFFLYSKLTVDKSRWQQGNVFSCSVMHEALHNHYTQKSLSLSPGK

SEQ ID NO: 52 - protein, 327 aa, synthetic construct
ASTKGPSVFPLAPCSRSTSESTAALGCLVKDYFPEPVTVSWNSGALTSGVHTFPAVLQSSGLYSLSSVVTVPSSSLGTKTYTCNVDHKPSNTKVDKRVESKYGPPCPSCPAPEFLGGPSVFLFPPKPKDTLMISRTPEVTCVVVDVSQEDPEVQFNWYVDGVEVHNAKTKPREEQFNSTYRVVSVLTVLHQDWLNGKEYKCKVSNKGLPSSIEKTISKAKGQPREPQVYTLPPSQEEMTKNQVSLTCLVKGFYPSDIAVEWESNGQPENNYKTTPPVLDSDGSFFLYSRLTVDKSRWQEGNVFSCSVMHEALHNHYTQKSLSLSLGK

SEQ ID NO: 53 - protein, 330 aa, synthetic construct
ASTKGPSVFPLAPSSKSTSGGTAALGCLVKDYFPEPVTVSWNSGALTSGVHTFPAVLQSSGLYSLSSVVTVPSSSLGTQTYICNVNHKPSNTKVDKKVEPKSCDKTHTCPPCPAPELLGGPDVFLFPPKPKDTLMISRTPEVTCVVVDVSHEDPEVKFNWYVDGVEVHNAKTKPREEQYNSTYRVVSVLTVLHQDWLNGKEYKCKVSNKALPLPEEKTISKAKGQPREPQVYTLPPSRDELTKNQVSLTCLVKGFYPSDIAVEWESNGQPENNYKTTPPVLDSDGSFFLYSKLTVDKSRWQQGNVFSCSVMHEALHNHYTQKSLSLSPGK

SEQ ID NO: 54 - protein, 440 aa, synthetic construct
QVQLVESGGGVVQPGRSLRLTCKASGLTFSSSGMHWVRQAPGKGLEWVAVIWYDGSKRYYADSVKGRFTISRDNSKNTLFLQMNSLRAEDTAVYYCATNNDYWGQGTLVTVSSASTKGPSVFPLAPCSRSTSESTAALGCLVKDYFPEPVTVSWNSGALTSGVHTFPAVLQSSGLYSLSSVVTVPSSSLGTKTYTCNVDHKPSNTKVDKRVESKYGPPCPPCPAPEFLGGPSVFLFPPKPKDTLMISRTPEVTCVVVDVSQEDPEVQFNWYVDGVEVHNAKTKPREEQFNSTYRVVSVLTVLHQDWLNGKEYKCKVSNKGLPSSIEKTISKAKGQPREPQVYTLPPSQEEMTKNQVSLTCLVKGFYPSDIAVEWESNGQPENNYKTTPPVLDSDGSFFLYSRLTVDKSRWQEGNVFSCSVMHEALHNHYTQKSLSLSLGK

SEQ ID NO: 55 - protein, 214 aa, synthetic construct
EIVLTQSPATLSLSPGERATLSCRASQSVSSYLAWYQQKPGQAPRLLIYTASNRATGIPARFSGSGSGTDFTLTISSLEPEDFAVYYCQQYSNWPRTFGQGTKVEIKRTVAAPSVFIFPPSDEQLKSGTASVVCLLNNFYPREAKVQWKVDNALQSGNSQESVTEQDSKDSTYSLSSTLTLSKADYEKHKVYACEVTHQGLSSPVTKSFNRGEC